European Patent Specification EP 3 962 923 B1, published April 19, 2023. Title: METHOD OF SEPARATION. Applicant: GE Healthcare Bioprocess R&D AB. The sequence listing filed with the application follows.

SEQUENCE LISTING (31 sequences)

SEQ ID NO: 1 - protein, 47 aa, Artificial Sequence
  Ligand consensus sequence
  misc_feature (3)..(3): Xaa can be any naturally occurring amino acid
  misc_feature (10)..(10): Xaa can be any naturally occurring amino acid
  misc_feature (20)..(20): Xaa can be any naturally occurring amino acid
  misc_feature (45)..(45): Xaa can be any naturally occurring amino acid
AQXAFYEILXLPNLTEEQRXAFIQSLKDDPSVSKAILAEAKKLNXAQ

SEQ ID NO: 2 - protein, 47 aa, Artificial Sequence
  Ligand example
AQEAFYEILHLPNLTEEQRNAFIQSLKDDPSVSKAILAEAKKLNDAQ

SEQ ID NO: 3 - protein, 47 aa, Artificial Sequence
  Ligand example
AQKAFYEILHLPNLTEEQRNAFIQSLKDDPSVSKAILAEAKKLNDAQ

SEQ ID NO: 4 - protein, 47 aa, Artificial Sequence
  Ligand example
AQEAFYEILKLPNLTEEQRNAFIQSLKDDPSVSKAILAEAKKLNDAQ

SEQ ID NO: 5 - protein, 47 aa, Artificial Sequence
  Ligand example
AQEAFYEILHLPNLTEEQRAAFIQSLKDDPSVSKAILAEAKKLNDAQ

SEQ ID NO: 6 - protein, 47 aa, Artificial Sequence
  Ligand example
AQEAFYEILHLPNLTEEQRNAFIQSLKDDPSVSKAILAEAKKLNWAQ

SEQ ID NO: 7 - protein, 352 aa, Artificial Sequence
  Hexameric ligand
AQGTVDAKFDKEAQEAFYEILHLPNLTEEQRNAFIQSLKDDPSVSKAILAEAKKLNDAQAPKVDAKFDKEAQEAFYEILHLPNLTEEQRNAFIQSLKDDPSVSKAILAEAKKLNDAQAPKVDAKFDKEAQEAFYEILHLPNLTEEQRNAFIQSLKDDPSVSKAILAEAKKLNDAQAPKVDAKFDKEAQEAFYEILHLPNLTEEQRNAFIQSLKDDPSVSKAILAEAKKLNDAQAPKVDAKFDKEAQEAFYEILHLPNLTEEQRNAFIQSLKDDPSVSKAILAEAKKLNDAQAPKVDAKFDKEAQEAFYEILHLPNLTEEQRNAFIQSLKDDPSVSKAILAEAKKLNDAQAPK

SEQ ID NO: 8 - protein, 11 aa, Artificial Sequence
  Linker
APKVDAKFDKE

SEQ ID NO: 9 - protein, 11 aa, Artificial Sequence
  Linker
APKVDNKFNKE

SEQ ID NO: 10 - protein, 11 aa, Artificial Sequence
  Linker
APKADNKFNKE

SEQ ID NO: 11 - protein, 8 aa, Artificial Sequence
  Linker
APKVFDKE

SEQ ID NO: 12 - protein, 8 aa, Artificial Sequence
  Linker
APAKFDKE

SEQ ID NO: 13 - protein, 6 aa, Artificial Sequence
  Linker
AKFDKE

SEQ ID NO: 14 - protein, 6 aa, Artificial Sequence
  Linker
APKVDA

SEQ ID NO: 15 - protein, 8 aa, Artificial Sequence
  Linker
VDAKFDKE

SEQ ID NO: 16 - protein, 8 aa, Artificial Sequence
  Linker
APKKFDKE

SEQ ID NO: 17 - protein, 15 aa, Artificial Sequence
  Linker
APKYEDGVDAKFDKE

SEQ ID NO: 18 - protein, 4 aa, Artificial Sequence
  Linker
YEDG

SEQ ID NO: 19 - protein, 4 aa, Artificial Sequence
  Leader
AQGT

SEQ ID NO: 20 - protein, 8 aa, Artificial Sequence
  Leader
VDAKFDKE

SEQ ID NO: 21 - protein, 10 aa, Artificial Sequence
  Leader
AQVDAKFDKE

SEQ ID NO: 22 - protein, 12 aa, Artificial Sequence
  Leader
AQGTVDAKFDKE

SEQ ID NO: 23 - protein, 138 aa, Artificial Sequence
  VHH
QVQLQESGGGLVQPGGSLRLSCAASGRTFSSYAMGWFRQAPGKQREFVAAIRWSGGYTYYTDSVKGRFTISRDNAKTTVYLQMNSLKPEDTAVYYCAATYLSSDYSRYALPQRPLDYDYWGQGTQVTVSSLEHHHHHH

SEQ ID NO: 24 - protein, 140 aa, Artificial Sequence
  VHH-EgA1
AQVDQLQESGGGLVQPGGSLRLSCAASGRTFSSYAMGWFRQAPGKQREFVAAIRWSGGYTYYTDSVKGRFTISRDNAKTTVYLQMNSLKPEDTAVYYCAATYLSSDYSRYALPQRPLDYDYWGQGTQVTVSSLEHHHHHH

SEQ ID NO: 25 - protein, 140 aa, Artificial Sequence
  VHH-EgA1 (T57K)
AQVDQLQESGGGLVQPGGSLRLSCAASGRTFSSYAMGWFRQAPGKQREFVAAIRWSGGYKYYTDSVKGRFTISRDNAKTTVYLQMNSLKPEDTAVYYCAATYLSSDYSRYALPQRPLDYDYWGQGTQVTVSSLEHHHHHH

SEQ ID NO: 26 - protein, 140 aa, Artificial Sequence
  VHH-EgA1 (T57K,K64R)
AQVDQLQESGGGLVQPGGSLRLSCAASGRTFSSYAMGWFRQAPGKQREFVAAIRWSGGYKYYTDSVRGRFTISRDNAKTTVYLQMNSLKPEDTAVYYCAATYLSSDYSRYALPQRPLDYDYWGQGTQVTVSSLEHHHHHH

SEQ ID NO: 27 - protein, 140 aa, Artificial Sequence
  VHH-EgA1 (T57P)
AQVDQLQESGGGLVQPGGSLRLSCAASGRTFSSYAMGWFRQAPGKQREFVAAIRWSGGYPYYTDSVKGRFTISRDNAKTTVYLQMNSLKPEDTAVYYCAATYLSSDYSRYALPQRPLDYDYWGQGTQVTVSSLEHHHHHH

SEQ ID NO: 28 - protein, 140 aa, Artificial Sequence
  VHH-EgA1 (T57S)
AQVDQLQESGGGLVQPGGSLRLSCAASGRTFSSYAMGWFRQAPGKQREFVAAIRWSGGYSYYTDSVKGRFTISRDNAKTTVYLQMNSLKPEDTAVYYCAATYLSSDYSRYALPQRPLDYDYWGQGTQVTVSSLEHHHHHH

SEQ ID NO: 29 - protein, 140 aa, Artificial Sequence
  VHH-EgA1 (T57R)
AQVDQLQESGGGLVQPGGSLRLSCAASGRTFSSYAMGWFRQAPGKQREFVAAIRWSGGYRYYTDSVKGRFTISRDNAKTTVYLQMNSLKPEDTAVYYCAATYLSSDYSRYALPQRPLDYDYWGQGTQVTVSSLEHHHHHH

SEQ ID NO: 30 - protein, 140 aa, Artificial Sequence
  VHH-EgA1 (S70T)
AQVDQLQESGGGLVQPGGSLRLSCAASGRTFSSYAMGWFRQAPGKQREFVAAIRWSGGYTYYTDSVKGRFTITRDNAKTTVYLQMNSLKPEDTAVYYCAATYLSSDYSRYALPQRPLDYDYWGQGTQVTVSSLEHHHHHH

SEQ ID NO: 31 - protein, 286 aa, Staphylococcus aureus
AQQNAFYQVLNMPNLNADQRNGFIQSLKDDPSQSANVLGEAQKLNDSQAPKADAQQNKFNKDQQSAFYEILNMPNLNEEQRNGFIQSLKDDPSQSTNVLGEAKKLNESQAPKADNNFNKEQQNAFYEILNMPNLNEEQRNGFIQSLKDDPSQSANLLAEAKKLNESQAPKADNKFNKEQQNAFYEILHLPNLNEEQRNGFIQSLKDDPSQSANLLAEAKKLNDAQAPKADNKFNKEQQNAFYEILHLPNLTEEQRNGFIQSLKDDPSVSKEILAEAKKLNDAQAPK